European Patent Specification EP 3 348 634 B1, published August 9, 2023. Title: A method of separating nucleic acids from a sample containing nucleic acids and a device for implementing the method. Applicant: Kaneka Corporation. The sequence listing filed with the application follows.

SEQUENCE LISTING (8 sequences)

SEQ ID NO: 1 - DNA, 20 bp, Artificial
  primer
acatgcaagtcgaacggaaa

SEQ ID NO: 2 - DNA, 20 bp, Artificial
  primer
cccaccaacaagctgatagg

SEQ ID NO: 3 - DNA, 20 bp, Artificial
  primer
acctcacctatgtgtcgacc

SEQ ID NO: 4 - DNA, 22 bp, Artificial
  primer
aacgtctttcaggtcgagtacg

SEQ ID NO: 5 - DNA, 25 bp, Artificial
  primer
ggaagaagcttgcttctttgctgac

SEQ ID NO: 6 - DNA, 26 bp, Artificial
  primer
agcccggggatttcacatctgactta

SEQ ID NO: 7 - DNA, 23 bp, Artificial
  primer
gctccactacaagatggacctgc

SEQ ID NO: 8 - DNA, 23 bp, Artificial
  primer
taggagtctgggccgtgtctcag